European Patent Application EP 4 431 528 A1, published September 18, 2024. Title: Isolated antigen binding protein and use thereof. Applicant: LONGBIO PHARMA (SUZHOU) CO., LTD. The sequence listing filed with the application follows.

SEQUENCE LISTING (82 sequences)

SEQ ID NO: 1 - protein, 6 aa, Artificial Sequence
  SE2/SE5/SE5ss heavy chain CDR1
SDYAWN

SEQ ID NO: 2 - protein, 16 aa, Artificial Sequence
  SE2/SE5ss heavy chain CDR2
YISYSGSTRYNPSLKS

SEQ ID NO: 3 - protein, 9 aa, Artificial Sequence
  SE2/SE5/SE5ss heavy chain CDR3
GSSQRFFDY

SEQ ID NO: 4 - protein, 30 aa, Artificial Sequence
  SE2/SE5 heavy chain FR1
DVQLLESGPGLVKPSQSLSLTCTVTGYSIT

SEQ ID NO: 5 - protein, 14 aa, Artificial Sequence
  SE2 heavy chain FR2
WIRQFPGNKLEWMG

SEQ ID NO: 6 - protein, 32 aa, Artificial Sequence
  SE2/SE5 heavy chain FR3
RISISRDTSKNQFFLQLNSVTSEDTATYFCVY

SEQ ID NO: 7 - protein, 11 aa, Artificial Sequence
  SE2/SE5 heavy chain FR4
WGQGTTLTVSS

SEQ ID NO: 8 - protein, 118 aa, Artificial Sequence
  SE2 heavy chain heavy chain variable region amino acid sequence
DVQLLESGPGLVKPSQSLSLTCTVTGYSITSDYAWNWIRQFPGNKLEWMGYISYSGSTRYNPSLKSRISISRDTSKNQFFLQLNSVTSEDTATYFCVYGSSQRFFDYWGQGTTLTVSS

SEQ ID NO: 9 - protein, 11 aa, Artificial Sequence
  SE2/SE5/SE5ss light chain CDR1
KASQDVSIDVA

SEQ ID NO: 10 - protein, 7 aa, Artificial Sequence
  SE2 light chain CDR2
SASFRYA

SEQ ID NO: 11 - protein, 8 aa, Artificial Sequence
  SE2 light chain CDR3
QQHYSLFT

SEQ ID NO: 12 - protein, 23 aa, Artificial Sequence
  SE2 light chain FR1
DILMTQSHKFMSTSIGDRVSITC

SEQ ID NO: 13 - protein, 15 aa, Artificial Sequence
  SE2 light chain FR2
WYHQKPGQSPKLLIY

SEQ ID NO: 14 - protein, 32 aa, Artificial Sequence
  SE2 light chain FR3
GVPDRFTGSGSGTDFTLTISSVQAEDLAVYYC

SEQ ID NO: 15 - protein, 10 aa, Artificial Sequence
  SE2/SE2 humanized/SE5 humanized/SE5ss humanized light chain FR4
FGSGTKLEIK

SEQ ID NO: 16 - protein, 106 aa, Artificial Sequence
  SE2 light chain variable region amino acid sequence
DILMTQSHKFMSTSIGDRVSITCKASQDVSIDVAWYHQKPGQSPKLLIYSASFRYAGVPDRFTGSGSGTDFTLTISSVQAEDLAVYYCQQHYSLFTFGSGTKLEIK

SEQ ID NO: 17 - protein, 30 aa, Artificial Sequence
  SE2 humanized/SE5 humanized/SE5ss humanized heavy chain FR1
QVQLQESGPGLVKPSQTLSLTCTVSGYSIT

SEQ ID NO: 18 - protein, 14 aa, Artificial Sequence
  SE2 humanized heavy chain FR2
WIRQPPGNGLEWMG

SEQ ID NO: 19 - protein, 32 aa, Artificial Sequence
  SE2 humanized/SE5 humanized/SE5ss humanized heavy chain FR3
RITISRDTSKNQFSLKLSSVTAADTAVYFCVY

SEQ ID NO: 20 - protein, 11 aa, Artificial Sequence
  SE2 humanized/SE5 humanized/SE5ss humanized heavy chain FR4
WGQGTLVTVSS

SEQ ID NO: 21 - protein, 118 aa, Artificial Sequence
  SE2 heavy chain variable region humanized amino acid sequence
QVQLQESGPGLVKPSQTLSLTCTVSGYSITSDYAWNWIRQPPGNGLEWMGYISYSGSTRYNPSLKSRITISRDTSKNQFSLKLSSVTAADTAVYFCVYGSSQRFFDYWGQGTLVTVSS

SEQ ID NO: 22 - protein, 23 aa, Artificial Sequence
  SE2 humanized light chain FR1
DILMTQSPDSLAVSLGERATINC

SEQ ID NO: 23 - protein, 15 aa, Artificial Sequence
  SE2 humanized/ SE5 humanized/SE5ss humanized light chain FR2
WYQQKPGQPPKLLIY

SEQ ID NO: 24 - protein, 32 aa, Artificial Sequence
  SE2 humanized light chain FR3
GVPDRFSGSGSGTDFTLTISSLQAEDVAVYYC

SEQ ID NO: 25 - protein, 106 aa, Artificial Sequence
  SE2 light chain variable region humanized amino acid sequence
DILMTQSPDSLAVSLGERATINCKASQDVSIDVAWYQQKPGQPPKLLIYSASFRYAGVPDRFSGSGSGTDFTLTISSLQAEDVAVYYCQQHYSLFTFGSGTKLEIK

SEQ ID NO: 26 - protein, 16 aa, Artificial Sequence
  SE5 heavy chain CDR2
YINYSGTTRYNPSLKS

SEQ ID NO: 27 - protein, 14 aa, Artificial Sequence
  SE5 heavy chain FR2
WIRQFPGNKLEWLG

SEQ ID NO: 28 - protein, 118 aa, Artificial Sequence
  SE5 heavy chain variable region amino acid sequence
DVQLLESGPGLVKPSQSLSLTCTVTGYSITSDYAWNWIRQFPGNKLEWLGYINYSGTTRYNPSLKSRISISRDTSKNQFFLQLNSVTSEDTATYFCVYGSSQRFFDYWGQGTTLTVSS

SEQ ID NO: 29 - protein, 7 aa, Artificial Sequence
  SE5/SE5ss light chain CDR2
SASWRYA

SEQ ID NO: 30 - protein, 8 aa, Artificial Sequence
  SE5/SE5ss light chain CDR3
QQHYNLFT

SEQ ID NO: 31 - protein, 23 aa, Artificial Sequence
  SE5 light chain FR1
DIVMTQSHKFMSTSVGDRVSITC

SEQ ID NO: 32 - protein, 15 aa, Artificial Sequence
  SE5 light chain FR2
WYQQKPGQSPKLLIY

SEQ ID NO: 33 - protein, 32 aa, Artificial Sequence
  SE5 light chain FR3
GVPDRFTGSRSGTDYTLTISSVQAEDLAVYYC

SEQ ID NO: 34 - protein, 10 aa, Artificial Sequence
  SE5 light chain FR4
FGSGTKLEIQ

SEQ ID NO: 35 - protein, 106 aa, Artificial Sequence
  SE5 light chain variable region amino acid sequence
DIVMTQSHKFMSTSVGDRVSITCKASQDVSIDVAWYQQKPGQSPKLLIYSASWRYAGVPDRFTGSRSGTDYTLTISSVQAEDLAVYYCQQHYNLFTFGSGTKLEIQ

SEQ ID NO: 36 - protein, 14 aa, Artificial Sequence
  SE5 humanized/SE5ss humanized heavy chain FR2
WIRQPPGNGLEWLG

SEQ ID NO: 37 - protein, 118 aa, Artificial Sequence
  SE5 heavy chain variable region humanized amino acid sequence
QVQLQESGPGLVKPSQTLSLTCTVSGYSITSDYAWNWIRQPPGNGLEWLGYINYSGTTRYNPSLKSRITISRDTSKNQFSLKLSSVTAADTAVYFCVYGSSQRFFDYWGQGTLVTVSS

SEQ ID NO: 38 - protein, 23 aa, Artificial Sequence
  SE5 humanized/SE5ss humanized light chain FR1
DIVMTQSPDSLAVSLGERATINC

SEQ ID NO: 39 - protein, 32 aa, Artificial Sequence
  SE5 humanized/SE5ss humanized light chain FR3
GVPDRFSGSRSGTDYTLTISSLQAEDVAVYYC

SEQ ID NO: 40 - protein, 106 aa, Artificial Sequence
  SE5 humanized/SE5ss humanized light chain variable region humanized amino acid sequence
DIVMTQSPDSLAVSLGERATINCKASQDVSIDVAWYQQKPGQPPKLLIYSASWRYAGVPDRFSGSRSGTDYTLTISSLQAEDVAVYYCQQHYNLFTFGSGTKLEIK

SEQ ID NO: 41 - protein, 118 aa, Artificial Sequence
  SE5ss heavy chain variable region humanized amino acid sequence
QVQLQESGPGLVKPSQTLSLTCTVSGYSITSDYAWNWIRQPPGNGLEWLGYISYSGSTRYNPSLKSRITISRDTSKNQFSLKLSSVTAADTAVYFCVYGSSQRFFDYWGQGTLVTVSS

SEQ ID NO: 42 - protein, 330 aa, Artificial Sequence [sequence omitted]

SEQ ID NO: 43 - protein, 107 aa, Artificial Sequence [sequence omitted]

SEQ ID NO: 44 - protein, 330 aa, Artificial Sequence
  SE5ss humanized heavy chain constant region amino acid sequence
ASTKGPSVFPLAPSSKSTSGGTAALGCLVKDYFPEPVTVSWNSGALTSGVHTFPAVLQSSGLYSLSSVVTVPSSSLGTQTYICNVNHKPSNTKVDKKVEPKSCDKTHTCPPCPAPEFQGGPSVFLFPPKPKDTLYITREPEVTCVVVDVSHEDPEVKFNWYVDGVEVHNAKTKPREEQYNSTYRVVSVLTVLHQDWLNGKEYKCQVSNKALPAPIEKTISKAKGQPREPQVYTLPPSRDELTKNQVSLTCLVKGFYPSDIAVEWESNGQPENNYKTTPPVLDSDGSFFLYSKLTVDKSRWQQGNVFSCSVMHEALHNHYTQKSLSLSPGK

SEQ ID NO: 45 - protein, 448 aa, Artificial Sequence
  SE2 humanized heavy chain complete sequence
QVQLQESGPGLVKPSQTLSLTCTVSGYSITSDYAWNWIRQPPGNGLEWMGYISYSGSTRYNPSLKSRITISRDTSKNQFSLKLSSVTAADTAVYFCVYGSSQRFFDYWGQGTLVTVSSASTKGPSVFPLAPSSKSTSGGTAALGCLVKDYFPEPVTVSWNSGALTSGVHTFPAVLQSSGLYSLSSVVTVPSSSLGTQTYICNVNHKPSNTKVDKKVEPKSCDKTHTCPPCPAPELLGGPSVFLFPPKPKDTLMISRTPEVTCVVVDVSHEDPEVKFNWYVDGVEVHNAKTKPREEQYNSTYRVVSVLTVLHQDWLNGKEYKCKVSNKALPAPIEKTISKAKGQPREPQVYTLPPSRDELTKNQVSLTCLVKGFYPSDIAVEWESNGQPENNYKTTPPVLDSDGSFFLYSKLTVDKSRWQQGNVFSCSVMHEALHNHYTQKSLSLSPGK

SEQ ID NO: 46 - protein, 213 aa, Artificial Sequence
  SE2 humanized light chain complete sequence
DILMTQSPDSLAVSLGERATINCKASQDVSIDVAWYQQKPGQPPKLLIYSASFRYAGVPDRFSGSGSGTDFTLTISSLQAEDVAVYYCQQHYSLFTFGSGTKLEIKRTVAAPSVFIFPPSDEQLKSGTASVVCLLNNFYPREAKVQWKVDNALQSGNSQESVTEQDSKDSTYSLSSTLTLSKADYEKHKVYACEVTHQGLSSPVTKSFNRGEC

SEQ ID NO: 47 - protein, 448 aa, Artificial Sequence
  SE5 humanized heavy chain complete sequence
QVQLQESGPGLVKPSQTLSLTCTVSGYSITSDYAWNWIRQPPGNGLEWLGYINYSGTTRYNPSLKSRITISRDTSKNQFSLKLSSVTAADTAVYFCVYGSSQRFFDYWGQGTLVTVSSASTKGPSVFPLAPSSKSTSGGTAALGCLVKDYFPEPVTVSWNSGALTSGVHTFPAVLQSSGLYSLSSVVTVPSSSLGTQTYICNVNHKPSNTKVDKKVEPKSCDKTHTCPPCPAPELLGGPSVFLFPPKPKDTLMISRTPEVTCVVVDVSHEDPEVKFNWYVDGVEVHNAKTKPREEQYNSTYRVVSVLTVLHQDWLNGKEYKCKVSNKALPAPIEKTISKAKGQPREPQVYTLPPSRDELTKNQVSLTCLVKGFYPSDIAVEWESNGQPENNYKTTPPVLDSDGSFFLYSKLTVDKSRWQQGNVFSCSVMHEALHNHYTQKSLSLSPGK

SEQ ID NO: 48 - protein, 213 aa, Artificial Sequence
  SE5 humanized/SE5ss humanized light chain complete sequence
DIVMTQSPDSLAVSLGERATINCKASQDVSIDVAWYQQKPGQPPKLLIYSASWRYAGVPDRFSGSRSGTDYTLTISSLQAEDVAVYYCQQHYNLFTFGSGTKLEIKRTVAAPSVFIFPPSDEQLKSGTASVVCLLNNFYPREAKVQWKVDNALQSGNSQESVTEQDSKDSTYSLSSTLTLSKADYEKHKVYACEVTHQGLSSPVTKSFNRGEC

SEQ ID NO: 49 - protein, 448 aa, Artificial Sequence
  SE5ss humanized heavy chain complete sequence
QVQLQESGPGLVKPSQTLSLTCTVSGYSITSDYAWNWIRQPPGNGLEWLGYISYSGSTRYNPSLKSRITISRDTSKNQFSLKLSSVTAADTAVYFCVYGSSQRFFDYWGQGTLVTVSSASTKGPSVFPLAPSSKSTSGGTAALGCLVKDYFPEPVTVSWNSGALTSGVHTFPAVLQSSGLYSLSSVVTVPSSSLGTQTYICNVNHKPSNTKVDKKVEPKSCDKTHTCPPCPAPEFQGGPSVFLFPPKPKDTLYITREPEVTCVVVDVSHEDPEVKFNWYVDGVEVHNAKTKPREEQYNSTYRVVSVLTVLHQDWLNGKEYKCQVSNKALPAPIEKTISKAKGQPREPQVYTLPPSRDELTKNQVSLTCLVKGFYPSDIAVEWESNGQPENNYKTTPPVLDSDGSFFLYSKLTVDKSRWQQGNVFSCSVMHEALHNHYTQKSLSLSPGK

SEQ ID NO: 50 - protein, 19 aa, Artificial Sequence
  Signal peptide amino acid sequence in the vector
MGWSCIILFLVATATGVHS

SEQ ID NO: 51 - protein, 405 aa, Artificial Sequence
  FCERIa-Fc protein amino acid sequence
VPQKPKVSLNPPWNRIFKGENVTLTCNGNNFFEVSSTKWFHNGSLSEETNSSLNIVNAKFEDSGEYKCQHQQVNESEPVYLEVFSDWLLLQASAEVVMEGQPLFLRCHGWRNWDVYKVIYYKDGEALKYWYENHNISITNATVEDSGTYYCTGKVWQLDYESEPLNITVIKAPEPKSCDKTHTCPPCPAPELLGGPSVFLFPPKPKDTLMISRTPEVTCVVVDVSHEDPEVKFNWYVDGVEVHNAKTKPREEQYNSTYRVVSVLTVLHQDWLNGKEYKCKVSNKALPAPIEKTISKAKGQPREPQVYTLPPSRDELTKNQVSLTCLVKGFYPSDIAVEWESNGQPENNYKTTPPVLDSDGSFFLYSKLTVDKSRWQQGNVFSCSVMHEALHNHYTQKSLSLSPGK

SEQ ID NO: 52 - protein, 325 aa, Artificial Sequence
  Fc region (CH2-4) amino acid sequence of human IgE
VCSRDFTPPTVKILQSSCDGGGHFPPTIQLLCLVSGYTPGTINITWLEDGQVMDVDLSTASTTQEGELASTQSELTLSQKHWLSDRTYTCQVTYQGHTFEDSTKKCADSNPRGVSAYLSRPSPFDLFIRKSPTITCLVVDLAPSKGTVNLTWSRASGKPVNHSTRKEEKQRNGTLTVTSTLPVGTRDWIEGETYQCRVTHPHLPRALMRSTTKTSGPRAAPEVYAFATPEWPGSRDKRTLACLIQNFMPEDISVQWLHNEVQLPDARHSTTQPRKTKGSGFFVFSRLEVTRAEWEQKDEFICRAVHEAASPSQTVQRAVSVNPGK

SEQ ID NO: 53 - DNA, 45 bp, Artificial Sequence
  Heavy chain /light chain variable region 5’ terminal primer 1
ctaatacgactcactatagggcaagcagtggtatcaacgcagagt

SEQ ID NO: 54 - DNA, 22 bp, Artificial Sequence
  Heavy chain /light chain variable region 5’ terminal primer 2
ctaatacgactcactatagggc

SEQ ID NO: 55 - DNA, 24 bp, Artificial Sequence
  Heavy chain variable region 3’ terminal primer
catcccagggtcaccatggagtta

SEQ ID NO: 56 - DNA, 24 bp, Artificial Sequence
  Light chain variable region 3’ terminal primer
gactgaggcacctccagatgttaa

SEQ ID NO: 57 - DNA, 408 bp, Artificial Sequence
  SE2 heavy chain variable region nucleotide sequence
atgagagtgctgattcttttgtggctgttcacagcctttcctggtttcctgtctgatgtgcagcttctggagtcgggacctggcctggtgaaaccttctcagtctctgtccctcacctgcactgtcactggctactcaatcaccagtgattatgcctggaactggatccggcagtttccaggaaacaaactggagtggatgggctacataagctacagtggtagtactaggtacaatccatctctcaaaagtcgaatttctatcagtcgagacacatccaagaaccagttcttcctgcagttgaattctgtgacttctgaggacacagccacatatttctgtgtttacggaagtagccagagattctttgactactggggccaaggcaccactctcacagtctcctca

SEQ ID NO: 58 - DNA, 405 bp, Artificial Sequence
  SE2 light chain variable region nucleotide sequence
atgcatcacaccagcatgggcatcaaaatggagtcacagattcaggtctttgtattcgtgtttctctggttgtctggtgttgacggagacattctgatgacccagtctcacaaattcatgtccacatcaattggagacagggtcagcatcacctgcaaggccagccaggatgtgagtattgatgtagcctggtatcaccagaaaccaggacaatctcctaaattactgatttactcggcttcgtttcggtacgctggagtccctgatcgcttcactggcagtggatctgggacggatttcactctcaccatcagcagtgtgcaggctgaagacctggcagtttattactgtcagcaacattatagtttattcacgttcggctcggggacaaagttggaaattaaa

SEQ ID NO: 59 - DNA, 354 bp, Artificial Sequence
  SE2 heavy chain variable region humanized nucleotide sequence
caggttcagctgcaagagtctggccctggcctggtcaagcctagccaaacactgagcctgacctgtaccgtgtccggctacagcatcaccagcgactacgcctggaactggatcagacagcctcctggcaatggactggaatggatgggctacatcagctacagcggcagcaccagatacaaccccagcctgaagtcccggatcaccatcagcagagacaccagcaagaaccagttctccctgaagctgagcagcgtgacagccgccgataccgccgtgtacttttgtgtgtacggcagcagccagcggttcttcgattattggggccagggcaccctggtcaccgtttcttct

SEQ ID NO: 60 - DNA, 318 bp, Artificial Sequence
  SE2 light chain variable region humanized nucleotide sequence
gacatcctgatgacacagagccctgatagcctggccgtgtctctgggagagagagccaccatcaattgcaaggccagccaggacgtgtccatcgacgtggcatggtatcagcagaagcctggccagcctcctaagctgctgatctacagcgccagcttcagatatgccggcgtgcccgatagattttccggctctggcagcggcaccgacttcacccttacaatcagttccctgcaggccgaggacgtggccgtgtactattgtcagcagcactacagcctgttcaccttcggctccggcaccaagctggaaatcaag

SEQ ID NO: 61 - DNA, 408 bp, Artificial Sequence
  SE5 heavy chain variable region nucleotide sequence
atgagagtgctgattcttttgtggctgttcacagcctttcctggtttcctgtctgatgtgcagcttctggagtcgggacctggcctggtgaaaccttctcagtctctgtccctcacctgcactgtcactggctactcaatcaccagtgattatgcctggaactggatccggcagtttccaggaaacaaattggagtggctgggctacataaactacagtggtaccactcgctacaatccatctctcaaaagtcgaatttctatcagtcgcgacacatccaagaaccagttcttcctgcagttgaattctgtgacttctgaggacacagccacatatttctgtgtttacggaagtagccagagattctttgactactggggccaaggcaccactctcacagtctcctca

SEQ ID NO: 62 - DNA, 414 bp, Artificial Sequence
  SE5 light chain variable region nucleotide sequence
atgggggaaatgcatcacaccagcatgggcatcaaaatggagtcacagattcaggtctttgtattcgtgtttctctggttgtctggtgttgacggagacattgtgatgacccagtctcacaaattcatgtccacatcagtaggagacagggtcagcatcacctgcaaggccagtcaggatgtgagtattgatgtagcctggtatcaacagaaaccaggacaatctcctaaactactgatttactcggcttcgtggcggtacgctggagtccctgatcgcttcactggcagtcgatctgggacggattatactctcaccatcagcagtgtgcaggctgaagacctggcagtttattactgtcagcaacattataatttattcacgttcggctcggggacaaagttggaaatacaa

SEQ ID NO: 63 - DNA, 354 bp, Artificial Sequence
  SE5 heavy chain variable region humanized nucleotide sequence
caggttcagctgcaagagtctggccctggcctggtcaagcctagccaaacactgagcctgacctgtaccgtgtccggctacagcatcaccagcgactacgcctggaactggatcagacagcctcctggcaatggactggaatggctgggctacatcaactacagcggcaccaccagatacaaccccagcctgaagtcccggatcaccatcagcagagacaccagcaagaaccagttctccctgaagctgagcagcgtgacagccgccgataccgccgtgtacttttgtgtgtacggcagcagccagcggttcttcgattattggggccagggcaccctggtcaccgtttcttct

SEQ ID NO: 64 - DNA, 318 bp, Artificial Sequence
  SE5 light chain variable region humanized nucleotide sequence
gacatcgtgatgacacagagccctgatagcctggccgtgtctctgggagagagagccaccatcaattgcaaggccagccaggacgtgtccatcgacgtggcatggtatcagcagaagcctggccagcctcctaagctgctgatctacagcgccagctggagatatgccggcgtgcccgatagattttccggctctagaagcggcaccgactatacccttacaatcagttccctgcaggccgaggacgtggccgtgtactattgtcagcagcactacaacctgttcaccttcggctccggcaccaagctggaaatcaag

SEQ ID NO: 65 - DNA, 354 bp, Artificial Sequence
  SE5ss heavy chain variable region humanized nucleotide sequence
caggtgcagctgcaggagagcggaccaggactggtgaagccaagccagaccctgtctctgacctgtacagtgagcggctactctatcacatccgactatgcctggaactggatcagacagccacctggaaatggactggagtggctgggctacatctcctatagcggctctacccgctacaatccaagcctgaagtctaggatcaccatctcccgggatacaagcaagaaccagttctccctgaagctgtccagcgtgaccgccgctgacacagccgtgtacttttgcgtgtatggctcttcccagaggttctttgattactggggccagggcaccctggtgacagtgagctct

SEQ ID NO: 66 - DNA, 318 bp, Artificial Sequence
  SE5ss light chain variable region humanized nucleotide sequence
gacatcgtgatgacccagtctccagattccctggccgtgtccctgggagagagggctacaatcaactgtaaggccagccaggacgtgtctatcgatgtggcctggtaccagcagaagcctggccagccccctaagctgctgatctactccgctagctggagatatgccggcgtgccagacaggttctctggctcccggagcggcaccgattacaccctgacaatctccagcctgcaggctgaggacgtggccgtgtactattgccagcagcactataatctgttcacctttggcagcggcacaaagctggagatcaag

SEQ ID NO: 67 - DNA, 1344 bp, Artificial Sequence
  Humanized SE2 heavy chain complete nucleotide sequence
caggttcagctgcaagagtctggccctggcctggtcaagcctagccaaacactgagcctgacctgtaccgtgtccggctacagcatcaccagcgactacgcctggaactggatcagacagcctcctggcaatggactggaatggatgggctacatcagctacagcggcagcaccagatacaaccccagcctgaagtcccggatcaccatcagcagagacaccagcaagaaccagttctccctgaagctgagcagcgtgacagccgccgataccgccgtgtacttttgtgtgtacggcagcagccagcggttcttcgattattggggccagggcaccctggtcaccgtttcttctgcgtcgaccaaaggcccctccgtgtttcctctggccccctcctccaagtctacctccggcggtaccgccgccctcggttgtttggtcaaagactacttccccgagcccgtgaccgtctcctggaactccggcgccctgacctccggcgtgcacacattccccgccgtcctgcagtcctccggcctgtactctctgtcttccgtggtgaccgtgccctccagctctttaggcacacagacctacatctgcaacgtgaaccacaagccctccaataccaaggtggacaagaaggtggagcccaagtcttgtgacaagacacacacttgtcctccttgtcccgctcccgaactgctgggaggccctagcgtgtttttattcccccctaaacctaaggacaccctcatgatcagccgtacccccgaagtgacttgtgtggtggtggacgtgtcccacgaggaccccgaagtcaagttcaactggtacgtggacggcgtggaggtgcataatgccaagaccaagccccgggaggagcagtataatagcacctatagggtggtgtccgtgctgaccgtgctgcaccaagattggctgaacggcaaggagtacaagtgtaaggtgtccaacaaggctttacccgctcccatcgagaagaccatctccaaggctaagggacagcctcgtgagcctcaagtttatactttacccccttctcgtgacgagctgaccaagaaccaagtttctttaacatgtttagtgaagggcttctacccctccgacatcgccgtggagtgggagagcaatggacagcccgagaacaactacaagaccacaccccccgttttagacagcgacggctccttctttttatactccaagctcaccgtggataagtcccggtggcagcaaggtaacgtcttctcttgttccgtgatgcacgaagctttacacaaccattacacccagaagtctttatctttaagccccggcaag

SEQ ID NO: 68 - DNA, 639 bp, Artificial Sequence
  Humanized SE2 light chain complete nucleotide sequence
gacatcctgatgacacagagccctgatagcctggccgtgtctctgggagagagagccaccatcaattgcaaggccagccaggacgtgtccatcgacgtggcatggtatcagcagaagcctggccagcctcctaagctgctgatctacagcgccagcttcagatatgccggcgtgcccgatagattttccggctctggcagcggcaccgacttcacccttacaatcagttccctgcaggccgaggacgtggccgtgtactattgtcagcagcactacagcctgttcaccttcggctccggcaccaagctggaaatcaagcgtacggtggctgcaccatctgtcttcatcttcccgccatctgatgagcagttgaaatctggaactgcctctgttgtgtgcctgctgaataacttctaccccagagaagccaaagtgcagtggaaggtggacaacgccctgcagagcggaaacagccaggaaagcgtgacagagcaggattccaaggattccacatacagcctgagcagcacactgacactgtccaaggccgactacgagaagcacaaggtgtacgcctgcgaagtgacacaccagggactgtcctcccctgtgacaaagagcttcaacagaggagaatgc

SEQ ID NO: 69 - DNA, 1344 bp, Artificial Sequence
  Humanized SE5 heavy chain complete nucleotide sequence
caggttcagctgcaagagtctggccctggcctggtcaagcctagccaaacactgagcctgacctgtaccgtgtccggctacagcatcaccagcgactacgcctggaactggatcagacagcctcctggcaatggactggaatggctgggctacatcaactacagcggcaccaccagatacaaccccagcctgaagtcccggatcaccatcagcagagacaccagcaagaaccagttctccctgaagctgagcagcgtgacagccgccgataccgccgtgtacttttgtgtgtacggcagcagccagcggttcttcgattattggggccagggcaccctggtcaccgtttcttctgcgtcgaccaaaggcccctccgtgtttcctctggccccctcctccaagtctacctccggcggtaccgccgccctcggttgtttggtcaaagactacttccccgagcccgtgaccgtctcctggaactccggcgccctgacctccggcgtgcacacattccccgccgtcctgcagtcctccggcctgtactctctgtcttccgtggtgaccgtgccctccagctctttaggcacacagacctacatctgcaacgtgaaccacaagccctccaataccaaggtggacaagaaggtggagcccaagtcttgtgacaagacacacacttgtcctccttgtcccgctcccgaactgctgggaggccctagcgtgtttttattcccccctaaacctaaggacaccctcatgatcagccgtacccccgaagtgacttgtgtggtggtggacgtgtcccacgaggaccccgaagtcaagttcaactggtacgtggacggcgtggaggtgcataatgccaagaccaagccccgggaggagcagtataatagcacctatagggtggtgtccgtgctgaccgtgctgcaccaagattggctgaacggcaaggagtacaagtgtaaggtgtccaacaaggctttacccgctcccatcgagaagaccatctccaaggctaagggacagcctcgtgagcctcaagtttatactttacccccttctcgtgacgagctgaccaagaaccaagtttctttaacatgtttagtgaagggcttctacccctccgacatcgccgtggagtgggagagcaatggacagcccgagaacaactacaagaccacaccccccgttttagacagcgacggctccttctttttatactccaagctcaccgtggataagtcccggtggcagcaaggtaacgtcttctcttgttccgtgatgcacgaagctttacacaaccattacacccagaagtctttatctttaagccccggcaag

SEQ ID NO: 70 - DNA, 639 bp, Artificial Sequence
  Humanized SE5 light chain complete nucleotide sequence
gacatcgtgatgacacagagccctgatagcctggccgtgtctctgggagagagagccaccatcaattgcaaggccagccaggacgtgtccatcgacgtggcatggtatcagcagaagcctggccagcctcctaagctgctgatctacagcgccagctggagatatgccggcgtgcccgatagattttccggctctagaagcggcaccgactatacccttacaatcagttccctgcaggccgaggacgtggccgtgtactattgtcagcagcactacaacctgttcaccttcggctccggcaccaagctggaaatcaagcgtacggtggctgcaccatctgtcttcatcttcccgccatctgatgagcagttgaaatctggaactgcctctgttgtgtgcctgctgaataacttctaccccagagaagccaaagtgcagtggaaggtggacaacgccctgcagagcggaaacagccaggaaagcgtgacagagcaggattccaaggattccacatacagcctgagcagcacactgacactgtccaaggccgactacgagaagcacaaggtgtacgcctgcgaagtgacacaccagggactgtcctcccctgtgacaaagagcttcaacagaggagaatgc

SEQ ID NO: 71 - DNA, 1344 bp, Artificial Sequence
  Humanized SE5ss heavy chain complete nucleotide sequence
caggtgcagctgcaggagagcggaccaggactggtgaagccaagccagaccctgtctctgacctgtacagtgagcggctactctatcacatccgactatgcctggaactggatcagacagccacctggaaatggactggagtggctgggctacatctcctatagcggctctacccgctacaatccaagcctgaagtctaggatcaccatctcccgggatacaagcaagaaccagttctccctgaagctgtccagcgtgaccgccgctgacacagccgtgtacttttgcgtgtatggctcttcccagaggttctttgattactggggccagggcaccctggtgacagtgagctctgcctctaccaagggcccctccgtgtttcctctggctccatccagcaagtccaccagcggaggaacagccgctctgggctgtctggtgaaggactatttccctgagccagtgaccgtgtcctggaacagcggcgccctgacctccggagtgcatacatttcccgctgtgctgcagtcttccggcctgtacagcctgagctctgtggtgaccgtgccttccagctctctgggcacccagacatatatctgcaacgtgaatcacaagccctctaatacaaaggtggacaagaaggtggagcctaagtcctgtgataagacccatacatgcccaccatgtccagctcctgagttccagggaggacctagcgtgttcctgtttcctccaaagccaaaggacaccctgtacatcacaagggagcctgaggtgacctgcgtggtggtggacgtgtctcacgaggatccagaggtgaagtttaactggtacgtggatggcgtggaggtgcataatgctaagaccaagcctagagaggagcagtacaatagcacctatcgcgtggtgtctgtgctgacagtgctgcaccaggactggctgaacggcaaggagtacaagtgccaggtgagcaataaggccctgccagctcccatcgagaagaccatctctaaggctaagggacagccaagggagcctcaggtgtacacactgcccccttcccgggacgagctgaccaagaaccaggtgagcctgacatgtctggtgaagggcttctatccaagcgatatcgctgtggagtgggagtctaatggccagcccgagaacaattacaagaccacaccacccgtgctggactctgatggctccttctttctgtattctaagctgaccgtggataagtcccggtggcagcagggcaacgtgttttcttgttccgtgatgcatgaggccctgcacaatcattatacacagaagagcctgtctctgtcccctggcaag

SEQ ID NO: 72 - DNA, 639 bp, Artificial Sequence
  Humanized SE5ss light chain complete nucleotide sequence
gacatcgtgatgacccagtctccagattccctggccgtgtccctgggagagagggctacaatcaactgtaaggccagccaggacgtgtctatcgatgtggcctggtaccagcagaagcctggccagccccctaagctgctgatctactccgctagctggagatatgccggcgtgccagacaggttctctggctcccggagcggcaccgattacaccctgacaatctccagcctgcaggctgaggacgtggccgtgtactattgccagcagcactataatctgttcacctttggcagcggcacaaagctggagatcaagagaaccgtggccgctcccagcgtgttcatctttccaccctctgacgagcagctgaagtccggcacagccagcgtggtgtgcctgctgaacaatttctaccctcgcgaggctaaggtgcagtggaaggtggataacgccctgcagagcggcaattctcaggagtccgtgaccgagcaggacagcaaggattctacatattccctgtcttccaccctgacactgtccaaggctgattacgagaagcacaaggtgtatgcctgcgaggtgacccatcagggcctgagctctcccgtgacaaagagctttaaccgcggcgagtgt

SEQ ID NO: 73 - protein, 118 aa, Artificial Sequence
  SE2/SE5 heavy chain variable region amino acid sequence general formula
  misc_feature (49)..(49): Xaa = Leu or Met
  misc_feature (53)..(53): Xaa = Asn or Ser
  misc_feature (57)..(57): Xaa = Ser or Thr
DVQLLESGPGLVKPSQSLSLTCTVTGYSITSDYAWNWIRQFPGNKLEWXGYIXYSGXTRYNPSLKSRISISRDTSKNQFFLQLNSVTSEDTATYFCVYGSSQRFFDYWGQGTTLTVSS

SEQ ID NO: 74 - protein, 118 aa, Artificial Sequence
  SE2/SE5/SE5ss heavy chain variable region humanized amino acid sequence general formula
  misc_feature (49)..(49): Xaa = Leu or Met
  misc_feature (53)..(53): Xaa = Asn or Ser
  misc_feature (57)..(57): Xaa = Ser or Thr
QVQLQESGPGLVKPSQTLSLTCTVSGYSITSDYAWNWIRQPPGNGLEWXGYIXYSGXTRYNPSLKSRITISRDTSKNQFSLKLSSVTAADTAVYFCVYGSSQRFFDYWGQGTLVTVSS

SEQ ID NO: 75 - protein, 106 aa, Artificial Sequence
  SE2/SE5 light chain variable region amino acid sequence general formula
  misc_feature (3)..(3): Xaa = Leu or Val
  misc_feature (15)..(15): Xaa = Ile or Val
  misc_feature (37)..(37): Xaa = His or Gln
  misc_feature (53)..(53): Xaa = Phe or Trp
  misc_feature (66)..(66): Xaa = Gly or Arg
  misc_feature (71)..(71): Xaa = Phe or Tyr
  misc_feature (93)..(93): Xaa = Asn or Ser
  misc_feature (106)..(106): Xaa = Lys or Gln
DIXMTQSHKFMSTSXGDRVSITCKASQDVSIDVAWYXQKPGQSPKLLIYSASXRYAGVPDRFTGSXSGTDXTLTISSVQAEDLAVYYCQQHYXLFTFGSGTKLEIX

SEQ ID NO: 76 - protein, 106 aa, Artificial Sequence
  SE2/SE5/SE5ss light chain variable region humanized amino acid sequence general formula
  misc_feature (3)..(3): Xaa = Leu or Val
  misc_feature (53)..(53): Xaa = Phe or Trp
  misc_feature (66)..(66): Xaa = Gly or Arg
  misc_feature (71)..(71): Xaa = Phe or Tyr
  misc_feature (93)..(93): Xaa = Asn or Ser
DIXMTQSPDSLAVSLGERATINCKASQDVSIDVAWYQQKPGQPPKLLIYSASXRYAGVPDRFSGSXSGTDXTLTISSLQAEDVAVYYCQQHYXLFTFGSGTKLEIK

SEQ ID NO: 77 - protein, 16 aa, Artificial Sequence
  SE2/SE5ss/SE5 heavy chain CDR2 general formula
  misc_feature (3)..(3): Xaa = Asn or Ser
  misc_feature (7)..(7): Xaa = Ser or Thr
YIXYSGXTRYNPSLKS

SEQ ID NO: 78 - protein, 7 aa, Artificial Sequence
  SE2/SE5/SE5ss light chain CDR2 general formula
  misc_feature (4)..(4): Xaa = Phe or Trp
SASXRYA

SEQ ID NO: 79 - protein, 8 aa, Artificial Sequence
  SE2/SE5/SE5ss light chain CDR3 general formula
  misc_feature (5)..(5): Xaa = Asn or Ser
QQHYXLFT

SEQ ID NO: 80 - protein, 23 aa, Artificial Sequence
  SE2/SE5/SE5ss light chain  humanized-FR1 general formula
  misc_feature (3)..(3): Xaa = Leu or Val
DIXMTQSPDSLAVSLGERATINC

SEQ ID NO: 81 - protein, 14 aa, Artificial Sequence
  SE2/SE5/SE5ss heavy chain  humanized-FR2 general formula
  misc_feature (13)..(13): Xaa = Leu or Met
WIRQPPGNGLEWXG

SEQ ID NO: 82 - protein, 32 aa, Artificial Sequence
  SE2/SE5/SE5ss light chain  humanized-FR3 general formula
  misc_feature (10)..(10): Xaa = Gly or Arg
  misc_feature (15)..(15): Xaa = Phe or Tyr
GVPDRFSGSXSGTDXTLTISSLQAEDVAVYYC